European Patent Specification EP 3 838 976 B1, published February 12, 2025. Title: PROCESS FOR DEGRADING PLASTIC PRODUCTS. Applicant: CARBIOS. The sequence listing filed with the application follows.

SEQUENCE LISTING (1 sequence)

SEQ ID NO: 1 - protein, 258 aa, ARTIFICIAL SEQUENCE
  CUTINASE
SNPYQRGPNPTRSALTADGPFSVATYTVSRLSVSGFGGGVIYYPTGTSLTFGGIAMSPGYTADASSLAWLGRRLASHGFVVLVINTNSRFDYPDSRASQLSAALNYLRTSSPSAVRARLDANRLAVAGHSMGGGGTLRIAEQNPSLKAAVPLTPWHTDKTFNTSVPVLIVGAEADTVAPVSQHAIPFYQNLPSTTPKVYVELDNASHFAPNSNNAAISVYTISWMKLWVDNDTRYRQFLCNVNDPALSDFRTNNRHCQ